European Patent Specification EP 3 197 914 B1, published February 7, 2024. Title: Anti-IL-25 Antibodies and Uses Thereof. Applicant: Regeneron Pharmaceuticals, Inc. The sequence listing filed with the application follows.

SEQUENCE LISTING (278 sequences)

SEQ ID NO: 1 - DNA, 363 bp, Artificial Sequence
  synthetic
gaggtgcagctggtggagtctgggggaggcttggtagagcctggggggtcccttagactctcctgtgtagcctctggattcactttcagtaacgcctggatgaactgggtccgccaggctccagggaaggggctggagtgggttggccatattgaaaggaaaactgatggtgggacaacagacttcgctgcacccgtgaaaggcagattcaccatctcaagagatgattcaaaaaacacgctgtatctgcaaatgaacagcctgaaaaccgaggacacagccgtgtattactgtaccacagtgggcccctacagtgtcccttttgactactggggccagggaaccctggtcaccgtctcctca

SEQ ID NO: 2 - protein, 121 aa, Artificial Sequence
  synthetic
EVQLVESGGGLVEPGGSLRLSCVASGFTFSNAWMNWVRQAPGKGLEWVGHIERKTDGGTTDFAAPVKGRFTISRDDSKNTLYLQMNSLKTEDTAVYYCTTVGPYSVPFDYWGQGTLVTVSS

SEQ ID NO: 3 - DNA, 24 bp, Artificial Sequence
  synthetic
ggattcactttcagtaacgcctgg

SEQ ID NO: 4 - protein, 8 aa, Artificial Sequence
  synthetic
GFTFSNAW

SEQ ID NO: 5 - DNA, 30 bp, Artificial Sequence
  synthetic
attgaaaggaaaactgatggtgggacaaca

SEQ ID NO: 6 - protein, 10 aa, Artificial Sequence
  synthetic
IERKTDGGTT

SEQ ID NO: 7 - DNA, 36 bp, Artificial Sequence
  synthetic
accacagtgggcccctacagtgtcccttttgactac

SEQ ID NO: 8 - protein, 12 aa, Artificial Sequence
  synthetic
TTVGPYSVPFDY

SEQ ID NO: 9 - DNA, 321 bp, Artificial Sequence
  synthetic
gacatccagatgacccagtctccatcctccctgtctgcatctgtaggagacagagtcaccatcacttgccgggcaagtcagagcattggcagctatttaaattggtatcagcagaaaccagggaaagcccctaagctcctgatctatgctgcatccagtttgcaaagtggggtcccatcaaggttcagtggcagtggatctgggacagatttcactctcaccatcagcagtctgcaacctgaagattttgcaacttactactgtcaacagacttacagtacccccatcaccttcggccaagggacacgactggagattaaa

SEQ ID NO: 10 - protein, 107 aa, Artificial Sequence
  synthetic
DIQMTQSPSSLSASVGDRVTITCRASQSIGSYLNWYQQKPGKAPKLLIYAASSLQSGVPSRFSGSGSGTDFTLTISSLQPEDFATYYCQQTYSTPITFGQGTRLEIK

SEQ ID NO: 11 - DNA, 18 bp, Artificial Sequence
  synthetic
cagagcattggcagctat

SEQ ID NO: 12 - protein, 6 aa, Artificial Sequence
  synthetic
QSIGSY

SEQ ID NO: 13 - DNA, 9 bp, Artificial Sequence
  synthetic
gctgcatcc

SEQ ID NO: 14 - protein, 3 aa, Artificial Sequence
  synthetic
AAS

SEQ ID NO: 15 - DNA, 27 bp, Artificial Sequence
  synthetic
caacagacttacagtacccccatcacc

SEQ ID NO: 16 - protein, 9 aa, Artificial Sequence
  synthetic
QQTYSTPIT

SEQ ID NO: 17 - DNA, 360 bp, Artificial Sequence
  synthetic
caggttcagctggtgcagtctggagctgaggtgaagaagcctggggcctcagtgaaggtctcctgcaaggcttctggttacacctttaccagctatggtatcagctgggtgcgacaggcccctggacaagggcttgagtggatgggatggatcagcgcttacaatggtaacacaaactatgcacagaagctccagggcagagtcaccatgaccacagacacatccacgagcacagcctacatggagctgaggagcctgagatctgacgacacggccgtgtattactgtgcgagagttcccataactggaactacctggttcgacccctggggccagggaaccctggtcaccgtctcctca

SEQ ID NO: 18 - protein, 120 aa, Artificial Sequence
  synthetic
QVQLVQSGAEVKKPGASVKVSCKASGYTFTSYGISWVRQAPGQGLEWMGWISAYNGNTNYAQKLQGRVTMTTDTSTSTAYMELRSLRSDDTAVYYCARVPITGTTWFDPWGQGTLVTVSS

SEQ ID NO: 19 - DNA, 24 bp, Artificial Sequence
  synthetic
ggttacacctttaccagctatggt

SEQ ID NO: 20 - protein, 8 aa, Artificial Sequence
  synthetic
GYTFTSYG

SEQ ID NO: 21 - DNA, 24 bp, Artificial Sequence
  synthetic
atcagcgcttacaatggtaacaca

SEQ ID NO: 22 - protein, 8 aa, Artificial Sequence
  synthetic
ISAYNGNT

SEQ ID NO: 23 - DNA, 39 bp, Artificial Sequence
  synthetic
gcgagagttcccataactggaactacctggttcgacccc

SEQ ID NO: 24 - protein, 13 aa, Artificial Sequence
  synthetic
ARVPITGTTWFDP

SEQ ID NO: 25 - DNA, 321 bp, Artificial Sequence
  synthetic
gacatccagatgacccagtctccatcctccctgtctgcatctgtaggagacagagtcaccatcacttgccgggcaagtcagagcattagcagctatttaaattggtatcagcagaaaccagggaaagcccctaagctcctgatctatgctgcatccagtttgcaaagtggggtcccatcaaggttcagtggcagtggatctgggacagatttcactctcaccatcagcagtctgcaacctgaagattttgcaacttactactgtcaacagacttacagtacccccatcaccttcggccaagggacacgactggagattaaa

SEQ ID NO: 26 - protein, 107 aa, Artificial Sequence
  synthetic
DIQMTQSPSSLSASVGDRVTITCRASQSISSYLNWYQQKPGKAPKLLIYAASSLQSGVPSRFSGSGSGTDFTLTISSLQPEDFATYYCQQTYSTPITFGQGTRLEIK

SEQ ID NO: 27 - DNA, 18 bp, Artificial Sequence
  synthetic
cagagcattagcagctat

SEQ ID NO: 28 - protein, 6 aa, Artificial Sequence
  synthetic
QSISSY

SEQ ID NO: 29 - DNA, 9 bp, Artificial Sequence
  synthetic
gctgcatcc

SEQ ID NO: 30 - protein, 3 aa, Artificial Sequence
  synthetic
AAS

SEQ ID NO: 31 - DNA, 27 bp, Artificial Sequence
  synthetic
caacagacttacagtacccccatcacc

SEQ ID NO: 32 - protein, 9 aa, Artificial Sequence
  synthetic
QQTYSTPIT

SEQ ID NO: 33 - DNA, 363 bp, Artificial Sequence
  synthetic
caggtgcagctgcaggagtcgggcccaggactggtgaagccttcggagaccctgtccctcacctgcactgtctctggtggctccatcagtagtcactactggagctggatccggcagcccccagggaagggactggaatggattggttttatctattacagtgggagcaccaacttcaacccctccctcaagagtcgagtcaccatttcaatagacacgtccaagaaccagttctccctgaagctgagctctgtgaccgccgcagacacggccgtgtattactgtgcgagacatgactacaatgactacgagctcaactacttcgatctctggggccgtggcaccctggcctctgtctcctca

SEQ ID NO: 34 - protein, 121 aa, Artificial Sequence
  synthetic
QVQLQESGPGLVKPSETLSLTCTVSGGSISSHYWSWIRQPPGKGLEWIGFIYYSGSTNFNPSLKSRVTISIDTSKNQFSLKLSSVTAADTAVYYCARHDYNDYELNYFDLWGRGTLASVSS

SEQ ID NO: 35 - DNA, 24 bp, Artificial Sequence
  synthetic
ggtggctccatcagtagtcactac

SEQ ID NO: 36 - protein, 8 aa, Artificial Sequence
  synthetic
GGSISSHY

SEQ ID NO: 37 - DNA, 21 bp, Artificial Sequence
  synthetic
atctattacagtgggagcacc

SEQ ID NO: 38 - protein, 7 aa, Artificial Sequence
  synthetic
IYYSGST

SEQ ID NO: 39 - DNA, 45 bp, Artificial Sequence
  synthetic
gcgagacatgactacaatgactacgagctcaactacttcgatctc

SEQ ID NO: 40 - protein, 15 aa, Artificial Sequence
  synthetic
ARHDYNDYELNYFDL

SEQ ID NO: 41 - DNA, 321 bp, Artificial Sequence; identical to SEQ ID NO: 25
  synthetic

SEQ ID NO: 42 - protein, 107 aa, Artificial Sequence; identical to SEQ ID NO: 26
  synthetic

SEQ ID NO: 43 - DNA, 18 bp, Artificial Sequence
  synthetic
cagagcattagcagctat

SEQ ID NO: 44 - protein, 6 aa, Artificial Sequence
  synthetic
QSISSY

SEQ ID NO: 45 - DNA, 9 bp, Artificial Sequence
  synthetic
gctgcatcc

SEQ ID NO: 46 - protein, 3 aa, Artificial Sequence
  synthetic
AAS

SEQ ID NO: 47 - DNA, 27 bp, Artificial Sequence
  synthetic
caacagacttacagtacccccatcacc

SEQ ID NO: 48 - protein, 9 aa, Artificial Sequence
  synthetic
QQTYSTPIT

SEQ ID NO: 49 - DNA, 363 bp, Artificial Sequence
  synthetic
caggtgcagctgcaggagtcgggcccaggtctggtgaagccttcggagaccctgtccctcacctgcactgtctctggtgcctccatcagtaattactactggagttggatccggcagcccccagggaagggactggagtggattggatatatcttttacagtgggaacaccaactacaacccctccctcaagagtcgagtcaccatttcagtagacacgtccaagaaccagttctccctgaagctgagctctgtgaccgccgcagacacggccgtgtattactgtgcgagagtcaggttcagtgactacgaactaaactggttcgacccctggggccaggggaccctggtcaccgtctcctca

SEQ ID NO: 50 - protein, 121 aa, Artificial Sequence
  synthetic
QVQLQESGPGLVKPSETLSLTCTVSGASISNYYWSWIRQPPGKGLEWIGYIFYSGNTNYNPSLKSRVTISVDTSKNQFSLKLSSVTAADTAVYYCARVRFSDYELNWFDPWGQGTLVTVSS

SEQ ID NO: 51 - DNA, 24 bp, Artificial Sequence
  synthetic
ggtgcctccatcagtaattactac

SEQ ID NO: 52 - protein, 8 aa, Artificial Sequence
  synthetic
GASISNYY

SEQ ID NO: 53 - DNA, 21 bp, Artificial Sequence
  synthetic
atcttttacagtgggaacacc

SEQ ID NO: 54 - protein, 7 aa, Artificial Sequence
  synthetic
IFYSGNT

SEQ ID NO: 55 - DNA, 45 bp, Artificial Sequence
  synthetic
gcgagagtcaggttcagtgactacgaactaaactggttcgacccc

SEQ ID NO: 56 - protein, 15 aa, Artificial Sequence
  synthetic
ARVRFSDYELNWFDP

SEQ ID NO: 57 - DNA, 339 bp, Artificial Sequence
  synthetic
gacatcgtgatgacccagtctccagactccctggctgtatttctgggcgagcgggccaccatcaactgcaggtccagccagagtgtttttctcggctccaacaataagaactacttagcttggtaccagcagaaacctggacagcctcctaaactactcatttactgggcgtcttcccgggaatccggggtccctgaccgattcagtggcagcgggtcagggacagatttcactctcactatcaacagcctgcaggctgaagatgtggcagtttattactgtcagcaatatttcattactccgctcactttcggcggagggaccaaggtggagatcaaa

SEQ ID NO: 58 - protein, 113 aa, Artificial Sequence
  synthetic
DIVMTQSPDSLAVFLGERATINCRSSQSVFLGSNNKNYLAWYQQKPGQPPKLLIYWASSRESGVPDRFSGSGSGTDFTLTINSLQAEDVAVYYCQQYFITPLTFGGGTKVEIK

SEQ ID NO: 59 - DNA, 36 bp, Artificial Sequence
  synthetic
cagagtgtttttctcggctccaacaataagaactac

SEQ ID NO: 60 - protein, 12 aa, Artificial Sequence
  synthetic
QSVFLGSNNKNY

SEQ ID NO: 61 - DNA, 9 bp, Artificial Sequence
  synthetic
tgggcgtct

SEQ ID NO: 62 - protein, 3 aa, Artificial Sequence
  synthetic
WAS

SEQ ID NO: 63 - DNA, 27 bp, Artificial Sequence
  synthetic
cagcaatatttcattactccgctcact

SEQ ID NO: 64 - protein, 9 aa, Artificial Sequence
  synthetic
QQYFITPLT

SEQ ID NO: 65 - DNA, 363 bp, Artificial Sequence
  synthetic
caggtgcagctgcaggagtcgggcccaggactggtgaagccttcggagaccctgtccctcacctgcactgtctctggtggctccatcagtagttacttctggagctggatccggcaggccccaggaaagggactggagtggattggatttatcgattacagtgggagcaccaactacaacccctccctcaagagtcgagtcaccatatcagtagacacgtccaagaaccagttctccctgaagttgaactctgtgaccgccgcagacacggccgtctattactgtgcgagacaagagatcattaacttcgagctgaactggttcgacccctggggccagggaaccctggtcactgtctcctca

SEQ ID NO: 66 - protein, 121 aa, Artificial Sequence
  synthetic
QVQLQESGPGLVKPSETLSLTCTVSGGSISSYFWSWIRQAPGKGLEWIGFIDYSGSTNYNPSLKSRVTISVDTSKNQFSLKLNSVTAADTAVYYCARQEIINFELNWFDPWGQGTLVTVSS

SEQ ID NO: 67 - DNA, 24 bp, Artificial Sequence
  synthetic
ggtggctccatcagtagttacttc

SEQ ID NO: 68 - protein, 8 aa, Artificial Sequence
  synthetic
GGSISSYF

SEQ ID NO: 69 - DNA, 21 bp, Artificial Sequence
  synthetic
atcgattacagtgggagcacc

SEQ ID NO: 70 - protein, 7 aa, Artificial Sequence
  synthetic
IDYSGST

SEQ ID NO: 71 - DNA, 45 bp, Artificial Sequence
  synthetic
gcgagacaagagatcattaacttcgagctgaactggttcgacccc

SEQ ID NO: 72 - protein, 15 aa, Artificial Sequence
  synthetic
ARQEIINFELNWFDP

SEQ ID NO: 73 - DNA, 339 bp, Artificial Sequence
  synthetic
gacatcgtgatgacccagtctccagcctccctggctgtgtctctgggcgagagggccaccatcaactgcaagtccagccagagtgttttatacagttccaacaataagaactacttagcttggtaccagcagaaaccaggacagcctcctaacctgctcatttactggtcatctacccgggactccggggtccctgaccgattcagtggcagcggttctggggcagatttcactctcaccatcagcagcctgcaggctgaagatgtggcagtttattactgtcagcaatattttagtactccgtggacgttcggccaagggaccaaggtggaaatcaaa

SEQ ID NO: 74 - protein, 113 aa, Artificial Sequence
  synthetic
DIVMTQSPASLAVSLGERATINCKSSQSVLYSSNNKNYLAWYQQKPGQPPNLLIYWSSTRDSGVPDRFSGSGSGADFTLTISSLQAEDVAVYYCQQYFSTPWTFGQGTKVEIK

SEQ ID NO: 75 - DNA, 36 bp, Artificial Sequence
  synthetic
cagagtgttttatacagttccaacaataagaactac

SEQ ID NO: 76 - protein, 12 aa, Artificial Sequence
  synthetic
QSVLYSSNNKNY

SEQ ID NO: 77 - DNA, 9 bp, Artificial Sequence
  synthetic
tggtcatct

SEQ ID NO: 78 - protein, 3 aa, Artificial Sequence
  synthetic
WSS

SEQ ID NO: 79 - DNA, 27 bp, Artificial Sequence
  synthetic
cagcaatattttagtactccgtggacg

SEQ ID NO: 80 - protein, 9 aa, Artificial Sequence
  synthetic
QQYFSTPWT

SEQ ID NO: 81 - DNA, 363 bp, Artificial Sequence
  synthetic
caggttcagctggtgcagtccggagctgaggtgaagaagcctggggcctcagtgaaggtctcctgtaaggcttctggttacacctttagtagttatggtattagctgggtgcgacaggcccctggacaagggcttgagtggatgggatggatcagcgcttacaatgataacacacagtatgcacagaaattccagggcagagtcaccatgaccacagacacatccacgagcacagcctacatggagctgaggagcctgagatctgacgacacggccgtgtattactgtgcgagagtcccattacaatggttcggggagtcctttgaccactggggccagggaaccctggtcaccgtctcctca

SEQ ID NO: 82 - protein, 121 aa, Artificial Sequence
  synthetic
QVQLVQSGAEVKKPGASVKVSCKASGYTFSSYGISWVRQAPGQGLEWMGWISAYNDNTQYAQKFQGRVTMTTDTSTSTAYMELRSLRSDDTAVYYCARVPLQWFGESFDHWGQGTLVTVSS

SEQ ID NO: 83 - DNA, 24 bp, Artificial Sequence
  synthetic
ggttacacctttagtagttatggt

SEQ ID NO: 84 - protein, 8 aa, Artificial Sequence
  synthetic
GYTFSSYG

SEQ ID NO: 85 - DNA, 24 bp, Artificial Sequence
  synthetic
atcagcgcttacaatgataacaca

SEQ ID NO: 86 - protein, 8 aa, Artificial Sequence
  synthetic
ISAYNDNT

SEQ ID NO: 87 - DNA, 42 bp, Artificial Sequence
  synthetic
gcgagagtcccattacaatggttcggggagtcctttgaccac

SEQ ID NO: 88 - protein, 14 aa, Artificial Sequence
  synthetic
ARVPLQWFGESFDH

SEQ ID NO: 89 - DNA, 321 bp, Artificial Sequence
  synthetic
gacatccagatgacccagtctccatcctccctgtctgcatctgtgggggacagagtcaccatcacttgccgggcaagtcaggacattaacaactatttaaattggtttcagcagaaaccagggaaagcccctaagctcctgatcttttctacatccagtttgcaaagtggggtcccatcaaggttcagtggcagtggctctggaacagatttcactctcaccatcagcagtctccaatctgaagattttgcaacttattactgtcaacagactttcattaccccgctcactttcggcggcgggaccaaggtggagatcaaa

SEQ ID NO: 90 - protein, 107 aa, Artificial Sequence
  synthetic
DIQMTQSPSSLSASVGDRVTITCRASQDINNYLNWFQQKPGKAPKLLIFSTSSLQSGVPSRFSGSGSGTDFTLTISSLQSEDFATYYCQQTFITPLTFGGGTKVEIK

SEQ ID NO: 91 - DNA, 18 bp, Artificial Sequence
  synthetic
caggacattaacaactat

SEQ ID NO: 92 - protein, 6 aa, Artificial Sequence
  synthetic
QDINNY

SEQ ID NO: 93 - DNA, 9 bp, Artificial Sequence
  synthetic
tctacatcc

SEQ ID NO: 94 - protein, 3 aa, Artificial Sequence
  synthetic
STS

SEQ ID NO: 95 - DNA, 27 bp, Artificial Sequence
  synthetic
caacagactttcattaccccgctcact

SEQ ID NO: 96 - protein, 9 aa, Artificial Sequence
  synthetic
QQTFITPLT

SEQ ID NO: 97 - DNA, 363 bp, Artificial Sequence
  synthetic
caggtgcagctgcaggagtcgggcccaggactggtgaagccttcggagaccctgtccctcacttgtactgtctctggtggctccatcagtaattacttctggagctggatccggcagcccccagggaagggactggagtggattgggtttaactataacagtgggagcaccaactataacccctccctcaagagtcgagtcaccatttcagtagacacgtccaagaaccagttctccctgaagctgagctctgtgaccgctgcggacacggccgtgtattactgtgcgagagggtataactggaactacgaaatagcttggttcgacccctggggccagggaaccctggtcactgtctcctca

SEQ ID NO: 98 - protein, 121 aa, Artificial Sequence
  synthetic
QVQLQESGPGLVKPSETLSLTCTVSGGSISNYFWSWIRQPPGKGLEWIGFNYNSGSTNYNPSLKSRVTISVDTSKNQFSLKLSSVTAADTAVYYCARGYNWNYEIAWFDPWGQGTLVTVSS

SEQ ID NO: 99 - DNA, 24 bp, Artificial Sequence
  synthetic
ggtggctccatcagtaattacttc

SEQ ID NO: 100 - protein, 8 aa, Artificial Sequence
  synthetic
GGSISNYF

SEQ ID NO: 101 - DNA, 21 bp, Artificial Sequence
  synthetic
aactataacagtgggagcacc

SEQ ID NO: 102 - protein, 7 aa, Artificial Sequence
  synthetic
NYNSGST

SEQ ID NO: 103 - DNA, 45 bp, Artificial Sequence
  synthetic
gcgagagggtataactggaactacgaaatagcttggttcgacccc

SEQ ID NO: 104 - protein, 15 aa, Artificial Sequence
  synthetic
ARGYNWNYEIAWFDP

SEQ ID NO: 105 - DNA, 321 bp, Artificial Sequence
  synthetic
gacatccagatgacccagtctccatcctccctgtctgcatctgtaggagacagagtcaccatcacttgccgggcaagtcagagcataagcagttatttaaattggtatcagcagaaaccagggaaagcccctaagctcctgatctatgctgcatccagtttgcaaagtggggtcccatcaaggttcagtggcagtggatctgggacagatttcactctcaccatcagcagtctgcaacctgaagattttgcaacttactattgtcaacagagttaccttaccccgctcactttcggcggagggaccaaggtggagatcaaa

SEQ ID NO: 106 - protein, 107 aa, Artificial Sequence
  synthetic
DIQMTQSPSSLSASVGDRVTITCRASQSISSYLNWYQQKPGKAPKLLIYAASSLQSGVPSRFSGSGSGTDFTLTISSLQPEDFATYYCQQSYLTPLTFGGGTKVEIK

SEQ ID NO: 107 - DNA, 18 bp, Artificial Sequence
  synthetic
cagagcataagcagttat

SEQ ID NO: 108 - protein, 6 aa, Artificial Sequence
  synthetic
QSISSY

SEQ ID NO: 109 - DNA, 9 bp, Artificial Sequence
  synthetic
gctgcatcc

SEQ ID NO: 110 - protein, 3 aa, Artificial Sequence
  synthetic
AAS

SEQ ID NO: 111 - DNA, 27 bp, Artificial Sequence
  synthetic
caacagagttaccttaccccgctcact

SEQ ID NO: 112 - protein, 9 aa, Artificial Sequence
  synthetic
QQSYLTPLT

SEQ ID NO: 113 - DNA, 375 bp, Artificial Sequence
  synthetic
caggttcagctggtgcagtctggagctgaggtgatgaagcctggggcctcagtgaaggtctcctgcaagtcttctgacttcgcctttaccacctatggcatcagctgggtgcgacaggcccctggacaagggcttgagtggatgggatggatcagcgcttacaatggtaacacaaactatgaacagaggttccagggcagaatcaccatgaccacagacacatccacgaccacagtttatatggagttgaggagcctgagatctgacgacacggccgtgtattactgtgcgagagatcccgactattgtagtagtaacacctgttctgatgcttttgatttgtggggccaagggacaatggtcaccgtctcttca

SEQ ID NO: 114 - protein, 125 aa, Artificial Sequence
  synthetic
QVQLVQSGAEVMKPGASVKVSCKSSDFAFTTYGISWVRQAPGQGLEWMGWISAYNGNTNYEQRFQGRITMTTDTSTTTVYMELRSLRSDDTAVYYCARDPDYCSSNTCSDAFDLWGQGTMVTVSS

SEQ ID NO: 115 - DNA, 24 bp, Artificial Sequence
  synthetic
gacttcgcctttaccacctatggc

SEQ ID NO: 116 - protein, 8 aa, Artificial Sequence
  synthetic
DFAFTTYG

SEQ ID NO: 117 - DNA, 24 bp, Artificial Sequence
  synthetic
atcagcgcttacaatggtaacaca

SEQ ID NO: 118 - protein, 8 aa, Artificial Sequence
  synthetic
ISAYNGNT

SEQ ID NO: 119 - DNA, 54 bp, Artificial Sequence
  synthetic
gcgagagatcccgactattgtagtagtaacacctgttctgatgcttttgatttg

SEQ ID NO: 120 - protein, 18 aa, Artificial Sequence
  synthetic
ARDPDYCSSNTCSDAFDL

SEQ ID NO: 121 - DNA, 321 bp, Artificial Sequence
  synthetic
gacatccagatgacccagtctccatcctccctgtctgcatctgtacgagacagagtcaccatcacttgccgggcgagtcagggcattaccaattatttagcctggtatcagcagaaaccagggaaagttcctaaggtcctgatctatgctgcatccactttgcaatcaggggtcccatctcggttcagtggcagtggctctgggacagaattcactctcgccatcagcagcctgcagcctgaggatgttgcaacttatttctgtcaacagtatggcagtgccccttggacgttcggccaagggaccaaggtggaaatcaaa

SEQ ID NO: 122 - protein, 107 aa, Artificial Sequence
  synthetic
DIQMTQSPSSLSASVRDRVTITCRASQGITNYLAWYQQKPGKVPKVLIYAASTLQSGVPSRFSGSGSGTEFTLAISSLQPEDVATYFCQQYGSAPWTFGQGTKVEIK

SEQ ID NO: 123 - DNA, 18 bp, Artificial Sequence
  synthetic
cagggcattaccaattat

SEQ ID NO: 124 - protein, 6 aa, Artificial Sequence
  synthetic
QGITNY

SEQ ID NO: 125 - DNA, 9 bp, Artificial Sequence
  synthetic
gctgcatcc

SEQ ID NO: 126 - protein, 3 aa, Artificial Sequence
  synthetic
AAS

SEQ ID NO: 127 - DNA, 27 bp, Artificial Sequence
  synthetic
caacagtatggcagtgccccttggacg

SEQ ID NO: 128 - protein, 9 aa, Artificial Sequence
  synthetic
QQYGSAPWT

SEQ ID NO: 129 - DNA, 360 bp, Artificial Sequence
  synthetic
caggttcagctggtgcagtctggagctgaggtgaagaaacctggggcctcagtgaaggtctcctgcaaggcttctgagtacacctttagcaactatggcatcagctgggtgcgacaggcccctggacaaggtcttgagtggttggggtggatcggcgcttatagtggtttcacaaaatatgcacagaaggtccaggacagaatcaccatgaccacagacgcatccacgaccacagcctacatggagctgagaaacctgagatctgacgacacggccgtgtattattgtgcgagagtgggaactggaactgactcttactttgacttctggggccagggaaccctggtcaccgtctcctca

SEQ ID NO: 130 - protein, 120 aa, Artificial Sequence
  synthetic
QVQLVQSGAEVKKPGASVKVSCKASEYTFSNYGISWVRQAPGQGLEWLGWIGAYSGFTKYAQKVQDRITMTTDASTTTAYMELRNLRSDDTAVYYCARVGTGTDSYFDFWGQGTLVTVSS

SEQ ID NO: 131 - DNA, 24 bp, Artificial Sequence
  synthetic
gagtacacctttagcaactatggc

SEQ ID NO: 132 - protein, 8 aa, Artificial Sequence
  synthetic
EYTFSNYG

SEQ ID NO: 133 - DNA, 24 bp, Artificial Sequence
  synthetic
atcggcgcttatagtggtttcaca

SEQ ID NO: 134 - protein, 8 aa, Artificial Sequence
  synthetic
IGAYSGFT

SEQ ID NO: 135 - DNA, 39 bp, Artificial Sequence
  synthetic
gcgagagtgggaactggaactgactcttactttgacttc

SEQ ID NO: 136 - protein, 13 aa, Artificial Sequence
  synthetic
ARVGTGTDSYFDF

SEQ ID NO: 137 - DNA, 321 bp, Artificial Sequence
  synthetic
gacatccagatgacccagtctccatcctccctgtctgcatctgtaggagacagagtcaccatcacttgccgggcaagtcagaacattaacagtcatttaaattggtatcagcagaaaccagggaaagcccctaaactcctgatttatactgcatccagtttgcaaagtggggtcccattaagattcagtggcagtggatctgggacagatttcactctcaccatcagcagtctgcaacctgaagattttggaatttacatctgtcaacagacttacataacccctctcactttcggcggtgggaccaaggtggagatcaaa

SEQ ID NO: 138 - protein, 107 aa, Artificial Sequence
  synthetic
DIQMTQSPSSLSASVGDRVTITCRASQNINSHLNWYQQKPGKAPKLLIYTASSLQSGVPLRFSGSGSGTDFTLTISSLQPEDFGIYICQQTYITPLTFGGGTKVEIK

SEQ ID NO: 139 - DNA, 18 bp, Artificial Sequence
  synthetic
cagaacattaacagtcat

SEQ ID NO: 140 - protein, 6 aa, Artificial Sequence
  synthetic
QNINSH

SEQ ID NO: 141 - DNA, 9 bp, Artificial Sequence
  synthetic
actgcatcc

SEQ ID NO: 142 - protein, 3 aa, Artificial Sequence
  synthetic
TAS

SEQ ID NO: 143 - DNA, 27 bp, Artificial Sequence
  synthetic
caacagacttacataacccctctcact

SEQ ID NO: 144 - protein, 9 aa, Artificial Sequence
  synthetic
QQTYITPLT

SEQ ID NO: 145 - DNA, 369 bp, Artificial Sequence
  synthetic
caggtgcagctgcaggagtcgggcccaggacttgtgaagtcttcggagaccctgtccctcacctgcactgtctctggtggctccatcagtagttactactggagctggatccggcagcccccagggaagggcctggaatggattggatttatctattacagtgggagcaccaactacaacccctccctcaagagtcgagtcaccttttcagtagacacttccaaaaaccacttctccctgaagctgaactctgtgaccgccacagacacggccgtgtattactgtgcgcgacattactttgattcggggacttatgaactggggccttttgactactggggccagggaaccctggtcaccgtctcctca

SEQ ID NO: 146 - protein, 123 aa, Artificial Sequence
  synthetic
QVQLQESGPGLVKSSETLSLTCTVSGGSISSYYWSWIRQPPGKGLEWIGFIYYSGSTNYNPSLKSRVTFSVDTSKNHFSLKLNSVTATDTAVYYCARHYFDSGTYELGPFDYWGQGTLVTVSS

SEQ ID NO: 147 - DNA, 24 bp, Artificial Sequence
  synthetic
ggtggctccatcagtagttactac

SEQ ID NO: 148 - protein, 8 aa, Artificial Sequence
  synthetic
GGSISSYY

SEQ ID NO: 149 - DNA, 21 bp, Artificial Sequence
  synthetic
atctattacagtgggagcacc

SEQ ID NO: 150 - protein, 7 aa, Artificial Sequence
  synthetic
IYYSGST

SEQ ID NO: 151 - DNA, 51 bp, Artificial Sequence
  synthetic
gcgcgacattactttgattcggggacttatgaactggggccttttgactac

SEQ ID NO: 152 - protein, 17 aa, Artificial Sequence
  synthetic
ARHYFDSGTYELGPFDY

SEQ ID NO: 153 - DNA, 339 bp, Artificial Sequence
  synthetic
gacatcgtgatgacccagtctccagactccctggctgtgtctctgggcgagagggccaccatcaactgcaagtccagccagaatattttattaacttccagtaataagaactacttaacttggtaccagcagaaaccaggacagcctcctaagctgctcatttactgggcatctattcgggaatccggggtccctgaccgattcagtggcagcgggtctgggacagatttcactctcaccatcagcagcctgcaggctgaagatgtggcactttatttctgtcagcaatattatattactccattcactttcggccctgggaccaaagtggatatcaaa

SEQ ID NO: 154 - protein, 113 aa, Artificial Sequence
  synthetic
DIVMTQSPDSLAVSLGERATINCKSSQNILLTSSNKNYLTWYQQKPGQPPKLLIYWASIRESGVPDRFSGSGSGTDFTLTISSLQAEDVALYFCQQYYITPFTFGPGTKVDIK

SEQ ID NO: 155 - DNA, 36 bp, Artificial Sequence
  synthetic
cagaatattttattaacttccagtaataagaactac

SEQ ID NO: 156 - protein, 12 aa, Artificial Sequence
  synthetic
QNILLTSSNKNY

SEQ ID NO: 157 - DNA, 9 bp, Artificial Sequence
  synthetic
tgggcatct

SEQ ID NO: 158 - protein, 3 aa, Artificial Sequence
  synthetic
WAS

SEQ ID NO: 159 - DNA, 27 bp, Artificial Sequence
  synthetic
cagcaatattatattactccattcact

SEQ ID NO: 160 - protein, 9 aa, Artificial Sequence
  synthetic
QQYYITPFT

SEQ ID NO: 161 - DNA, 372 bp, Artificial Sequence
  synthetic
caggtgcagctgcaggagtcgggcccaggactggtgaagccttcggagaccctgtccctcacctgcactgtctctggtggctccatcagtgattactactggagctggatccggcagcccccagggaagggactggagtggattggccatatctattacagtgggagcaccaaccacaacccctccctcaagagtcgagtcgccatatcagtcgacacgtccaagaaccagttctccctgaggctgtactctgtgaccgctgcggacacggccgtgtattactgtgcgagagacgggtatagtagctcgtccggcttctactacttcggtatggacgtctggggccaagggaccacggtcaccgtctcctca

SEQ ID NO: 162 - protein, 124 aa, Artificial Sequence
  synthetic
QVQLQESGPGLVKPSETLSLTCTVSGGSISDYYWSWIRQPPGKGLEWIGHIYYSGSTNHNPSLKSRVAISVDTSKNQFSLRLYSVTAADTAVYYCARDGYSSSSGFYYFGMDVWGQGTTVTVSS

SEQ ID NO: 163 - DNA, 24 bp, Artificial Sequence
  synthetic
ggtggctccatcagtgattactac

SEQ ID NO: 164 - protein, 8 aa, Artificial Sequence
  synthetic
GGSISDYY

SEQ ID NO: 165 - DNA, 21 bp, Artificial Sequence
  synthetic
atctattacagtgggagcacc

SEQ ID NO: 166 - protein, 7 aa, Artificial Sequence
  synthetic
IYYSGST

SEQ ID NO: 167 - DNA, 54 bp, Artificial Sequence
  synthetic
gcgagagacgggtatagtagctcgtccggcttctactacttcggtatggacgtc

SEQ ID NO: 168 - protein, 18 aa, Artificial Sequence
  synthetic
ARDGYSSSSGFYYFGMDV

SEQ ID NO: 169 - DNA, 321 bp, Artificial Sequence
  synthetic
gacatccagttgacccagtctccatccttcctgtctgcatctgtcggagacagagtcaccatcacttgctgggccagtcaggacattaacagttatttagcctggtatcagcaaaaaccagggaaagcccctaagctcctgatctttgctgcatccactttgcaaggtggggtcccttctaggttcagcggcagtggatctgggacagaattcactctcacaatcagcagcctgcagcctgaagattttgcaacttattactgtcaacaccttagtagtttccctcccaccttcggccaagggacacgactggagattaaa

SEQ ID NO: 170 - protein, 107 aa, Artificial Sequence
  synthetic
DIQLTQSPSFLSASVGDRVTITCWASQDINSYLAWYQQKPGKAPKLLIFAASTLQGGVPSRFSGSGSGTEFTLTISSLQPEDFATYYCQHLSSFPPTFGQGTRLEIK

SEQ ID NO: 171 - DNA, 18 bp, Artificial Sequence
  synthetic
caggacattaacagttat

SEQ ID NO: 172 - protein, 6 aa, Artificial Sequence
  synthetic
QDINSY

SEQ ID NO: 173 - DNA, 9 bp, Artificial Sequence
  synthetic
gctgcatcc

SEQ ID NO: 174 - protein, 3 aa, Artificial Sequence
  synthetic
AAS

SEQ ID NO: 175 - DNA, 27 bp, Artificial Sequence
  synthetic
caacaccttagtagtttccctcccacc

SEQ ID NO: 176 - protein, 9 aa, Artificial Sequence
  synthetic
QHLSSFPPT

SEQ ID NO: 177 - DNA, 363 bp, Artificial Sequence
  synthetic
caggtgcagctgcaggagtcgggcccaggactggtgaggccttcggagaccctatccctcatctgcactgtctctggtggctccatcaatagttactactggagctggatccggcagcccccagggaagggactggaatggattggatatatctattacagtgggagcaccaactacaacccctccctcaagagtcgagtcaccatatcaggagacacgtccaagaaccagttctccctgaagctgagctctgtgaccgctgcggacacggccgtgtattactgcgcgagaggggtaatctggaactacgaactccgagaatttgactactggggccagggaaccctggtcaccgtctcctca

SEQ ID NO: 178 - protein, 121 aa, Artificial Sequence
  synthetic
QVQLQESGPGLVRPSETLSLICTVSGGSINSYYWSWIRQPPGKGLEWIGYIYYSGSTNYNPSLKSRVTISGDTSKNQFSLKLSSVTAADTAVYYCARGVIWNYELREFDYWGQGTLVTVSS

SEQ ID NO: 179 - DNA, 24 bp, Artificial Sequence
  synthetic
ggtggctccatcaatagttactac

SEQ ID NO: 180 - protein, 8 aa, Artificial Sequence
  synthetic
GGSINSYY

SEQ ID NO: 181 - DNA, 21 bp, Artificial Sequence
  synthetic
atctattacagtgggagcacc

SEQ ID NO: 182 - protein, 7 aa, Artificial Sequence
  synthetic
IYYSGST

SEQ ID NO: 183 - DNA, 45 bp, Artificial Sequence
  synthetic
gcgagaggggtaatctggaactacgaactccgagaatttgactac

SEQ ID NO: 184 - protein, 15 aa, Artificial Sequence
  synthetic
ARGVIWNYELREFDY

SEQ ID NO: 185 - DNA, 339 bp, Artificial Sequence
  synthetic
gacatcgtgatgacccagtctccagactccctggctgtgtctctgggcgagagggccaccatcaactgcaagtccagccagagtgttttagacagttccaacaataagaactacttagtttggtaccagcagaaaccaggacagcctcctgagctgctcatttactgggcatctacccgggaatccggggtccctgaccgattcagtggcagcgggtctgggacagatttcactctcaccatcagcagcctgcaggctgaagatgtggcagtttattactgtcagcaatattattttactccgctcaccttcggcggagggaccaaggtggagatcaaa

SEQ ID NO: 186 - protein, 113 aa, Artificial Sequence
  synthetic
DIVMTQSPDSLAVSLGERATINCKSSQSVLDSSNNKNYLVWYQQKPGQPPELLIYWASTRESGVPDRFSGSGSGTDFTLTISSLQAEDVAVYYCQQYYFTPLTFGGGTKVEIK

SEQ ID NO: 187 - DNA, 36 bp, Artificial Sequence
  synthetic
cagagtgttttagacagttccaacaataagaactac

SEQ ID NO: 188 - protein, 12 aa, Artificial Sequence
  synthetic
QSVLDSSNNKNY

SEQ ID NO: 189 - DNA, 9 bp, Artificial Sequence
  synthetic
tgggcatct

SEQ ID NO: 190 - protein, 3 aa, Artificial Sequence
  synthetic
WAS

SEQ ID NO: 191 - DNA, 27 bp, Artificial Sequence
  synthetic
cagcaatattattttactccgctcacc

SEQ ID NO: 192 - protein, 9 aa, Artificial Sequence
  synthetic
QQYYFTPLT

SEQ ID NO: 193 - DNA, 369 bp, Artificial Sequence
  synthetic
cagctgcagctgcaggagtcgggcccaggactggtgaggccttcggagaccctgtccctcacctgcagtgtctcgagtggctccatcagaagtagtaattactactggggctggatccgccagcccccagggaagggactggagtggattgggaatatctattatagtgggaacaccttctataacccgtccctcaagggtcgagtcaccatatccgtagacacgtccaagaaccagttctccctgaagctgagctctgtgaccgccacagacacggctgtgtattactgtgcgagacaaggatatagtgactacgagttgaactggttcgacccctggggccagggaaccctggtcaccgtctcctca

SEQ ID NO: 194 - protein, 123 aa, Artificial Sequence
  synthetic
QLQLQESGPGLVRPSETLSLTCSVSSGSIRSSNYYWGWIRQPPGKGLEWIGNIYYSGNTFYNPSLKGRVTISVDTSKNQFSLKLSSVTATDTAVYYCARQGYSDYELNWFDPWGQGTLVTVSS

SEQ ID NO: 195 - DNA, 30 bp, Artificial Sequence
  synthetic
agtggctccatcagaagtagtaattactac

SEQ ID NO: 196 - protein, 10 aa, Artificial Sequence
  synthetic
SGSIRSSNYY

SEQ ID NO: 197 - DNA, 21 bp, Artificial Sequence
  synthetic
atctattatagtgggaacacc

SEQ ID NO: 198 - protein, 7 aa, Artificial Sequence
  synthetic
IYYSGNT

SEQ ID NO: 199 - DNA, 45 bp, Artificial Sequence
  synthetic
gcgagacaaggatatagtgactacgagttgaactggttcgacccc

SEQ ID NO: 200 - protein, 15 aa, Artificial Sequence
  synthetic
ARQGYSDYELNWFDP

SEQ ID NO: 201 - DNA, 339 bp, Artificial Sequence
  synthetic
gacatcgtgatgacccagtctccagactccctggtgctgtctctgggcgagagggccaccttcaactgcaagtccagccagagtgttttagacagttccaacaataagaactacttagcttggtaccagcagaaaccaggacagcctcctaagttgctcatttactgggcatctacccgggaatccggggtccctgaccgattcagtggcagcgggtctgggacagatttctctctcaccatcagcagcctgcaggctgaagatgtggcactttattactgtcaacaattttataatagtccgtggacgttcggccaagggaccaaggtggaaatcaaa

SEQ ID NO: 202 - protein, 113 aa, Artificial Sequence
  synthetic
DIVMTQSPDSLVLSLGERATFNCKSSQSVLDSSNNKNYLAWYQQKPGQPPKLLIYWASTRESGVPDRFSGSGSGTDFSLTISSLQAEDVALYYCQQFYNSPWTFGQGTKVEIK

SEQ ID NO: 203 - DNA, 36 bp, Artificial Sequence; identical to SEQ ID NO: 187
  synthetic

SEQ ID NO: 204 - protein, 12 aa, Artificial Sequence
  synthetic
QSVLDSSNNKNY

SEQ ID NO: 205 - DNA, 9 bp, Artificial Sequence
  synthetic
tgggcatct

SEQ ID NO: 206 - protein, 3 aa, Artificial Sequence
  synthetic
WAS

SEQ ID NO: 207 - DNA, 27 bp, Artificial Sequence
  synthetic
caacaattttataatagtccgtggacg

SEQ ID NO: 208 - protein, 9 aa, Artificial Sequence
  synthetic
QQFYNSPWT

SEQ ID NO: 209 - DNA, 363 bp, Artificial Sequence
  synthetic
caggtgcagctgcaggagtcgggcccagggctggtgaagccctcggagaccctgtccctcacctgcactgtctctggtggctccatcaatagttattcttggacctggatccggcagcccccagggaagggactggaatggattggaaatatctataatagtgagaataccaactacaacccctccctcaagagtcgagtcaccatatcagttgacacgtccaagagtcaggtttccctgaaactgaactctgtgaccgctgcggacacggccgtatattactgtgcgagaacatataactggaactacgaaataggggccatgggcgtctggggccaggggaccacggtcaccgtctcctca

SEQ ID NO: 210 - protein, 121 aa, Artificial Sequence
  synthetic
QVQLQESGPGLVKPSETLSLTCTVSGGSINSYSWTWIRQPPGKGLEWIGNIYNSENTNYNPSLKSRVTISVDTSKSQVSLKLNSVTAADTAVYYCARTYNWNYEIGAMGVWGQGTTVTVSS

SEQ ID NO: 211 - DNA, 24 bp, Artificial Sequence
  synthetic
ggtggctccatcaatagttattct

SEQ ID NO: 212 - protein, 8 aa, Artificial Sequence
  synthetic
GGSINSYS

SEQ ID NO: 213 - DNA, 21 bp, Artificial Sequence
  synthetic
atctataatagtgagaatacc

SEQ ID NO: 214 - protein, 7 aa, Artificial Sequence
  synthetic
IYNSENT

SEQ ID NO: 215 - DNA, 45 bp, Artificial Sequence
  synthetic
gcgagaacatataactggaactacgaaataggggccatgggcgtc

SEQ ID NO: 216 - protein, 15 aa, Artificial Sequence
  synthetic
ARTYNWNYEIGAMGV

SEQ ID NO: 217 - DNA, 339 bp, Artificial Sequence
  synthetic
gacatcgtgatgacccagtttccagactccctggctgtgtctctgggcgagagggccaccatcaactgcaagtccagccagaatgttttaatcacctccaacaataagaattatttagcttggtaccagcagaaaccaggacagcctcctaagctgctcatttactgggcttccacccgggaattcggggtccctgcccgattcagtggcagcgggtctgggacagatttcactctcaccatcagcagcctgcaggctgaagatgtggcagtttattactgtcagcaatattatagtactccattcactttcggccctgggaccaaagtggatatcaaa

SEQ ID NO: 218 - protein, 113 aa, Artificial Sequence
  synthetic
DIVMTQFPDSLAVSLGERATINCKSSQNVLITSNNKNYLAWYQQKPGQPPKLLIYWASTREFGVPARFSGSGSGTDFTLTISSLQAEDVAVYYCQQYYSTPFTFGPGTKVDIK

SEQ ID NO: 219 - DNA, 36 bp, Artificial Sequence
  synthetic
cagaatgttttaatcacctccaacaataagaattat

SEQ ID NO: 220 - protein, 12 aa, Artificial Sequence
  synthetic
QNVLITSNNKNY

SEQ ID NO: 221 - DNA, 9 bp, Artificial Sequence
  synthetic
tgggcttcc

SEQ ID NO: 222 - protein, 3 aa, Artificial Sequence
  synthetic
WAS

SEQ ID NO: 223 - DNA, 27 bp, Artificial Sequence
  synthetic
cagcaatattatagtactccattcact

SEQ ID NO: 224 - protein, 9 aa, Artificial Sequence
  synthetic
QQYYSTPFT

SEQ ID NO: 225 - DNA, 363 bp, Artificial Sequence
  synthetic
caggttcagctggtgcagtctggagctgaggtgaagaagcctgggacctcagtgaaggtctcctgcaaggcttctggttacacctttaccaactatggtatcagttgggtgcgacaggcccctggacaaggtcttgagtggttgggatggatcagcgcttataatgataacacagactatgcacagaaactccaggccagagtcaccatgaccacagacacattcacgagcacagcctacatggacctgaggagcctgagatctgacgacacggccgtgtattactgtgcgagagttcctataactggaactacctcaagttttgacttctggggccagggaaccctggtcaccgtctcctca

SEQ ID NO: 226 - protein, 121 aa, Artificial Sequence
  synthetic
QVQLVQSGAEVKKPGTSVKVSCKASGYTFTNYGISWVRQAPGQGLEWLGWISAYNDNTDYAQKLQARVTMTTDTFTSTAYMDLRSLRSDDTAVYYCARVPITGTTSSFDFWGQGTLVTVSS

SEQ ID NO: 227 - DNA, 24 bp, Artificial Sequence
  synthetic
ggttacacctttaccaactatggt

SEQ ID NO: 228 - protein, 8 aa, Artificial Sequence
  synthetic
GYTFTNYG

SEQ ID NO: 229 - DNA, 24 bp, Artificial Sequence
  synthetic
atcagcgcttataatgataacaca

SEQ ID NO: 230 - protein, 8 aa, Artificial Sequence
  synthetic
ISAYNDNT

SEQ ID NO: 231 - DNA, 42 bp, Artificial Sequence
  synthetic
gcgagagttcctataactggaactacctcaagttttgacttc

SEQ ID NO: 232 - protein, 14 aa, Artificial Sequence
  synthetic
ARVPITGTTSSFDF

SEQ ID NO: 233 - DNA, 321 bp, Artificial Sequence
  synthetic
gacatccagatgacccagtctccatcctccctgtctgcatctgtaggagacagagtcaccatctcttgccgggcaagtcagaccatttacagctatttaaattggtttcagcagaaaccagggaaagcccctaagctcctgatctatgatgcatccagtttgcaaagtggggtcccatcaaggttcagtggcagtggctctgggacacatttcactctcaccatcagcagtctgcaacctgaggattttgcaacttacttctgccaacagacttacagtacccctctcactttcggcggagggaccaaggtggagatcaaa

SEQ ID NO: 234 - protein, 107 aa, Artificial Sequence
  synthetic
DIQMTQSPSSLSASVGDRVTISCRASQTIYSYLNWFQQKPGKAPKLLIYDASSLQSGVPSRFSGSGSGTHFTLTISSLQPEDFATYFCQQTYSTPLTFGGGTKVEIK

SEQ ID NO: 235 - DNA, 18 bp, Artificial Sequence
  synthetic
cagaccatttacagctat

SEQ ID NO: 236 - protein, 6 aa, Artificial Sequence
  synthetic
QTIYSY

SEQ ID NO: 237 - DNA, 9 bp, Artificial Sequence
  synthetic
gatgcatcc

SEQ ID NO: 238 - protein, 3 aa, Artificial Sequence
  synthetic
DAS

SEQ ID NO: 239 - DNA, 27 bp, Artificial Sequence
  synthetic
caacagacttacagtacccctctcact

SEQ ID NO: 240 - protein, 9 aa, Artificial Sequence
  synthetic
QQTYSTPLT

SEQ ID NO: 241 - DNA, 360 bp, Artificial Sequence
  synthetic
caggtgcagctgcaggagtcgggcccaggactggtgaaaccttcggagaccctgtccctcacctgcactgtctctggtggctccatcagtagttactactggagctggatccggcagcccccagggaagggactggagtggattggctttatctattacagtgggagcaccaactacaacccctccctcaagagtcgagtcaccatctcagtagacacgtccaagaaccagttctccctgaagctgagttctgtgaccgccgcagacacggccgtgtattactgtgcgagacatgacagtgactacgaactctacggtatggacgtctggggccaagggaccacggtcaccgtctcctca

SEQ ID NO: 242 - protein, 120 aa, Artificial Sequence
  synthetic
QVQLQESGPGLVKPSETLSLTCTVSGGSISSYYWSWIRQPPGKGLEWIGFIYYSGSTNYNPSLKSRVTISVDTSKNQFSLKLSSVTAADTAVYYCARHDSDYELYGMDVWGQGTTVTVSS

SEQ ID NO: 243 - DNA, 24 bp, Artificial Sequence
  synthetic
ggtggctccatcagtagttactac

SEQ ID NO: 244 - protein, 8 aa, Artificial Sequence
  synthetic
GGSISSYY

SEQ ID NO: 245 - DNA, 21 bp, Artificial Sequence
  synthetic
atctattacagtgggagcacc

SEQ ID NO: 246 - protein, 7 aa, Artificial Sequence
  synthetic
IYYSGST

SEQ ID NO: 247 - DNA, 42 bp, Artificial Sequence
  synthetic
gcgagacatgacagtgactacgaactctacggtatggacgtc

SEQ ID NO: 248 - protein, 14 aa, Artificial Sequence
  synthetic
ARHDSDYELYGMDV

SEQ ID NO: 249 - DNA, 339 bp, Artificial Sequence
  synthetic
gacatcgtgatgacccagtctccagactccctggctgtgtctctgggcgagagggccaccatcacctgcaagtccagccagagtattttatacaactccgacaataagaactacttagcttggtaccagcagaaatcaggacagcctcctaagctgctcatttcctgggcatctacccgggaatccggggtccctgaccgtttcagtggcagcgggtctgggacagatttcactctcaccatcagcagcctgcaggctgaagatgtggcagtttattactgtcaacaatatttttttactccattcactttcggccctgggaccaaagtggatatcaaa

SEQ ID NO: 250 - protein, 113 aa, Artificial Sequence
  synthetic
DIVMTQSPDSLAVSLGERATITCKSSQSILYNSDNKNYLAWYQQKSGQPPKLLISWASTRESGVPDRFSGSGSGTDFTLTISSLQAEDVAVYYCQQYFFTPFTFGPGTKVDIK

SEQ ID NO: 251 - DNA, 36 bp, Artificial Sequence
  synthetic
cagagtattttatacaactccgacaataagaactac

SEQ ID NO: 252 - protein, 12 aa, Artificial Sequence
  synthetic
QSILYNSDNKNY

SEQ ID NO: 253 - DNA, 9 bp, Artificial Sequence
  synthetic
tgggcatct

SEQ ID NO: 254 - protein, 3 aa, Artificial Sequence
  synthetic
WAS

SEQ ID NO: 255 - DNA, 27 bp, Artificial Sequence
  synthetic
caacaatatttttttactccattcact

SEQ ID NO: 256 - protein, 9 aa, Artificial Sequence
  synthetic
QQYFFTPFT

SEQ ID NO: 257 - DNA, 363 bp, Artificial Sequence
  synthetic
gaggtgcagctggtggagtctgggggaggcttggtacagcctggggggtccctgagactctcctgtgcagcctctggattcaccttcagtaactacgacatacactgggtccgccaagttccaggaaaaggtctggagtggatctcaactattggttctgctggtgatacattctatccaggctccgtgaagggccggttcaccatctccagagaaaatgccaagaactccctgtatcttcaaatgaacagcctgagagccggggactcggctgtatattactgtgcaagaggggataactggaactacgtttcatggttcttcgatctctggggccgtggcaccctggtcactgtctcctca

SEQ ID NO: 258 - protein, 121 aa, Artificial Sequence
  synthetic
EVQLVESGGGLVQPGGSLRLSCAASGFTFSNYDIHWVRQVPGKGLEWISTIGSAGDTFYPGSVKGRFTISRENAKNSLYLQMNSLRAGDSAVYYCARGDNWNYVSWFFDLWGRGTLVTVSS

SEQ ID NO: 259 - DNA, 24 bp, Artificial Sequence
  synthetic
ggattcaccttcagtaactacgac

SEQ ID NO: 260 - protein, 8 aa, Artificial Sequence
  synthetic
GFTFSNYD

SEQ ID NO: 261 - DNA, 21 bp, Artificial Sequence
  synthetic
attggttctgctggtgataca

SEQ ID NO: 262 - protein, 7 aa, Artificial Sequence
  synthetic
IGSAGDT

SEQ ID NO: 263 - DNA, 45 bp, Artificial Sequence
  synthetic
gcaagaggggataactggaactacgtttcatggttcttcgatctc

SEQ ID NO: 264 - protein, 15 aa, Artificial Sequence
  synthetic
ARGDNWNYVSWFFDL

SEQ ID NO: 265 - DNA, 321 bp, Artificial Sequence
  synthetic
gacatccagttgacccagtctccatccttcctgtctacatctgtcggagacagagtcaccatcacgtgctgggccagtcaggacatcagcagttttttagcctggtatcagcagaaaccagggaaagcccctaaactcctgatctatgctgcgtccgttttgcaaagtggggtcccatcaaggttcagcggcagtggatctgggacagaattcactctcacaatcagcagtctgcagcctgaagattttgcaacttattactgtcagcaggttaatagttacccgatcaccttcggccaagggacacgactggagattaaa

SEQ ID NO: 266 - protein, 107 aa, Artificial Sequence
  synthetic
DIQLTQSPSFLSTSVGDRVTITCWASQDISSFLAWYQQKPGKAPKLLIYAASVLQSGVPSRFSGSGSGTEFTLTISSLQPEDFATYYCQQVNSYPITFGQGTRLEIK

SEQ ID NO: 267 - DNA, 18 bp, Artificial Sequence
  synthetic
caggacatcagcagtttt

SEQ ID NO: 268 - protein, 6 aa, Artificial Sequence
  synthetic
QDISSF

SEQ ID NO: 269 - DNA, 9 bp, Artificial Sequence
  synthetic
gctgcgtcc

SEQ ID NO: 270 - protein, 3 aa, Artificial Sequence
  synthetic
AAS

SEQ ID NO: 271 - DNA, 27 bp, Artificial Sequence
  synthetic
cagcaggttaatagttacccgatcacc

SEQ ID NO: 272 - protein, 9 aa, Artificial Sequence
  synthetic
QQVNSYPIT

SEQ ID NO: 273 - protein, 173 aa, Artificial Sequence
  hIL-25-MMH aa 1-145: hIL-25 (aa 33-177 of NP_073626.1) aa 146-173: myc-myc-hexahistidine tag
YSHWPSCCPSKGQDTSEELLRWSTVPVPPLEPARPNRHPESCRASEDGPLNSRAISPWRYELDRDLNRLPQDLYHARCLCPHCVSLQTGSHMDPRGNSELLYHNQTVFYRRPCHGEKGTHKGYCLERRLYRVSLACVCVRPRVMGEQKLISEEDLGGEQKLISEEDLHHHHHH

SEQ ID NO: 274 - protein, 172 aa, Artificial Sequence
  MfIL-25-MMH aa 1-144: M.fascicularis IL-25 (aa 33-176 of XP_001107906.2) aa 145-172: myc-myc-hexahistidine tag
YSHWPSCCPSKGYPSEELLRWSTVPVPPLKPASLDFHSVSCRASEDGPLNSRAISPWRYELDRDLNRLPQDLYHARCLCPHCVSLQTGSHMDPRGNSELLYHNQTVFYRRPCHGKKGNHKGYCLERRLYRVSLACVCVRPRVMGEQKLISEEDLGGEQKLISEEDLHHHHHH

SEQ ID NO: 275 - protein, 181 aa, Artificial Sequence
  mouse IL-25-MMH aa 1-153: Mouse IL-25 (aa 17-169 of  NP_542767.1) aa 154-181: myc-myc-hexahistidine tag
VSLRIQEGCSHLPSCCPSKEQEPPEEWLKWSSASVSPPEPLSHTHHAESCRASKDGPLNSRAISPWSYELDRDLNRVPQDLYHARCLCPHCVSLQTGSHMDPLGNSVPLYHNQTVFYRRPCHGEEGTHRRYCLERRLYRVSLACVCVRPRVMAEQKLISEEDLGGEQKLISEEDLHHHHHH

SEQ ID NO: 276 - protein, 181 aa, Artificial Sequence
  rat IL-25-MMH aa 1-153: Rat IL-25 (aa 17-169 of NP_001178936.1) aa 154-181: myc-myc-hexahistidine tag
VSLRIQEDCSHLPRCCPSKQQEFPEEWLKWNPAPVSPPEPLRHTHHPESCRASKDGPLNSRAISPWSYELDRDLNRVPQDLYHARCLCPHCVSLQTGSHMDPMGNSVPLYHNQTVFYRRPCHGEQGAHGRYCLERRLYRVSLACVCVRPRMMAEQKLISEEDLGGEQKLISEEDLHHHHHH

SEQ ID NO: 277 - DNA, 1335 bp, Artificial Sequence
  Human IL-25 (NM_022789.3)
ggcttgctgaaaataaaatcaggactcctaacctgctccagtcagcctgcttccacgaggcctgtcagtcagtgccccacttgtgactgagtgtgcagtgcccagcatgtaccaggtcagtgcagagggctgcctgagggctgtgctgagagggagaggagcagagatgctgctgagggtggagggaggccaagctgccaggtttggggctgggggccaagtggagtgagaaactgggatcccagggggagggtgcagatgagggagcgacccagattaggtgaggacagttctctcattagccttttcctacaggtggttgcattcttggcaatggtcatgggaacccacacctacagccactggcccagctgctgccccagcaaagggcaggacacctctgaggagctgctgaggtggagcactgtgcctgtgcctcccctagagcctgctaggcccaaccgccacccagagtcctgtagggccagtgaagatggacccctcaacagcagggccatctccccctggagatatgagttggacagagacttgaaccggctcccccaggacctgtaccacgcccgttgcctgtgcccgcactgcgtcagcctacagacaggctcccacatggacccccggggcaactcggagctgctctaccacaaccagactgtcttctaccggcggccatgccatggcgagaagggcacccacaagggctactgcctggagcgcaggctgtaccgtgtttccttagcttgtgtgtgtgtgcggccccgtgtgatgggctagccggacctgctggaggctggtccctttttgggaaacctggagccaggtgtacaaccacttgccatgaagggccaggatgcccagatgcttggcccctgtgaagtgctgtctggagcagcaggatcccgggacaggatggggggctttggggaaagcctgcacttctgcacattttgaaaagagcagctgctgcttagggccgccggaagctggtgtcctgtcattttctctcaggaaaggttttcaaagttctgcccatttctggaggccaccactcctgtctcttcctcttttcccatcccctgctaccctggcccagcacaggcactttctagatatttcccccttgctggagaagaaagagcccctggttttatttgtttgtttactcatcactcagtgagcatctactttgggtgcattctagtgtagttactagtcttttgacatggatgattctgaggaggaagctgttattgaatgtatagagatttatccaaataaatatctttatttaaaaatgaaaaaaaaaaaaaaaaaaaa

SEQ ID NO: 278 - protein, 177 aa, Artificial Sequence
  Human IL-25
MRERPRLGEDSSLISLFLQVVAFLAMVMGTHTYSHWPSCCPSKGQDTSEELLRWSTVPVPPLEPARPNRHPESCRASEDGPLNSRAISPWRYELDRDLNRLPQDLYHARCLCPHCVSLQTGSHMDPRGNSELLYHNQTVFYRRPCHGEKGTHKGYCLERRLYRVSLACVCVRPRVMG